European Patent Application EP 4 663 658 A1, published December 17, 2025. Title: Single-domain antibody specifically binding to CLL1 protein and use thereof. Applicant: CARBIOGENE THERAPEUTICS CO.,LTD. Application CN. The sequence listing filed with the application follows.

SEQUENCE LISTING (4 sequences)

SEQ ID NO: 1 - protein, 129 aa, synthetic construct
DVQLQESGGGLVQPGGSLRLSCAASGFTFGDYDMTWVRQAPGKGPEWVSAINSGGGSTYYADSVKGRFTISRDNAKNTLYLQMNSLKPEDTAVYYCATIDRLSTVVAGTYQPSDEYDYWGQGTQVTVSS

SEQ ID NO: 2 - DNA, 387 bp, synthetic construct
  source 1..387: mol_type = other DNA
gatgtgcagctgcaggagtctggaggaggcttggtgcagcctgggggttctctgagactctcctgtgcagcctctggattcaccttcggagactatgacatgacctgggtccgccaggctccaggaaaggggcccgagtgggtctcagctattaatagtggcggtggtagcacatactatgcagactccgtgaagggccgattcaccatctccagagacaacgccaagaacacgctgtatctgcaaatgaacagcctgaaacctgaggacacggccgtgtattactgtgcaactatcgaccgccttagtacggtagtagctggtacgtaccagccgtccgatgagtatgactactggggccaggggacccaggtcaccgtctccagc

SEQ ID NO: 3 - DNA, 696 bp, Homo sapiens
  source 1..696: mol_type = genomic DNA
gagcccaaatctgctgacaaaactcacacatgcccaccgtgcccagcacctgaactcctggggggaccgtcagtcttcctcttccccccaaaacccaaggacaccctcatgatctcccggacccccgaggtcacatgcgtggtggtggacgtgagccacgaagaccctgaggtcaagttcaactggtacgtggacggcgtggaggtgcataatgccaagacaaagccgcgggaggagcagtacaacagcacgtaccgtgtggtcagcgtcctcaccgtcctgcaccaggactggctgaatggcaaggagtacaagtgcaaggtctccaacaaagccctcccagcccccatcgagaaaaccatctccaaagccaaagggcagccccgagaaccacaggtgtacaccctgcccccatcccgggaggagatgaccaagaaccaggtcagcctgacctgcctggtcaaaggcttctatcccagcgacatcgccgtggagtgggagagcaatgggcagccggagaacaactacaagaccacgcctcccgtgctggactccgacggctccttcttcctctacagcaagctcaccgtggacaagagcaggtggcagcaggggaacgtcttctcatgctccgtgatgcatgaggctctgcacaaccactacacgcagaagagcctctccctgtctccgggtaaa

SEQ ID NO: 4 - protein, 232 aa, Homo sapiens
EPKSADKTHTCPPCPAPELLGGPSVFLFPPKPKDTLMISRTPEVTCVVVDVSHEDPEVKFNWYVDGVEVHNAKTKPREEQYNSTYRVVSVLTVLHQDWLNGKEYKCKVSNKALPAPIEKTISKAKGQPREPQVYTLPPSREEMTKNQVSLTCLVKGFYPSDIAVEWESNGQPENNYKTTPPVLDSDGSFFLYSKLTVDKSRWQQGNVFSCSVMHEALHNHYTQKSLSLSPGK